European Patent Application EP 4 699 658 A2, published February 25, 2026. Title: METHODS AND COMPOSITIONS FOR TREATING SKELETAL MUSCULAR DYSTROPHY. Applicant: Cedars-Sinai Medical Center. The sequence listing filed with the application follows.

SEQUENCE LISTING (6 sequences)

SEQ ID NO: 1 - RNA, 68 nt, Homo sapiens
  source 1..68: mol_type = unassigned RNA
gaggcaaagttctgagacactccgactctgagtatgatagaagtcagtgcactacagaactttgtctc

SEQ ID NO: 2 - RNA, 22 nt, Homo sapiens
  source 1..22: mol_type = unassigned RNA
aaagttctgagacactccgact

SEQ ID NO: 3 - RNA, 22 nt, Homo sapiens
  source 1..22: mol_type = unassigned RNA
tcagtgcactacagaactttgt

SEQ ID NO: 4 - RNA, 115 nt, Homo sapiens
  source 1..115: mol_type = unassigned RNA
tgtacacagaggctgatcgattctccctgaacagcctattacggaggcactgcagatcaagcccgcctggagaggtggagtttcaagagtcccttcctggttcaccgtctccttt

SEQ ID NO: 5 - RNA, 113 nt, Homo sapiens
  source 1..113: mol_type = unassigned RNA
tgtacacggtggagtttcaagagtcccttcctggttcaccgtctcctttagaggctgatcgattctccctgaacagcctattacggaggcactgcagatcaagcccgcctgga

SEQ ID NO: 6 - RNA, 115 nt, Homo sapiens
  source 1..115: mol_type = unassigned RNA
tccccacagaggctgatcgattctccctgaacagcctcctccggaggcactgcagatcaagcccgcctggagaggtggagtttcaagagtcccttcctggttcaccgtctccttt